European Patent Application EP 4 428 247 A1, published September 11, 2024. Title: Method of Amplification or Detection of Target Material using Nanoparticles. Applicant: Seoul National University R&DB Foundation. The sequence listing filed with the application follows.

SEQUENCE LISTING (8 sequences)

SEQ ID NO: 1 - DNA, 30 bp, synthetic construct
  misc_feature 1..30: note = Target strand
  source 1..30: mol_type = other DNA
gagggattattgttaaatattgataaggat

SEQ ID NO: 2 - DNA, 45 bp, synthetic construct
  misc_feature 1..45: note = Template strand
  source 1..45: mol_type = other DNA
taacaataatccctcatccttatcaatatttaacaataatccctc

SEQ ID NO: 3 - DNA, 15 bp, synthetic construct
  misc_feature 1..15: note = Magnetic particle strand (target-capturing strand)
  source 1..15: mol_type = other DNA
atccttatcaatatt

SEQ ID NO: 4 - DNA, 30 bp, synthetic construct
  misc_feature 1..30: note = Toehold strand
  source 1..30: mol_type = other DNA
atccttatcaatatttaacaataatccctc

SEQ ID NO: 5 - DNA, 30 bp, synthetic construct
  misc_feature 1..30: note = Single-base mismatch strand
  source 1..30: mol_type = other DNA
gagggattattgttaaatatttataaggat

SEQ ID NO: 6 - DNA, 30 bp, synthetic construct
  misc_feature 1..30: note = Nonspecific strand
  source 1..30: mol_type = other DNA
ctgattactattgcatcttccgttacaact

SEQ ID NO: 7 - DNA, 18 bp, synthetic construct
  misc_feature 1..18: note = F-primer
  source 1..18: mol_type = other DNA
ctggctcaggatgaacgc

SEQ ID NO: 8 - DNA, 18 bp, synthetic construct
  misc_feature 1..18: note = R-primer
  source 1..18: mol_type = other DNA
cgacttcgggtgttacaa